European Patent Application EP 4 530 351 A2, published April 2, 2025. Title: COMPOSITIONS AND METHODS FOR IMPROVED GENE EDITING. Applicant: ASTRAZENECA AB. The sequence listing filed with the application follows.

SEQUENCE LISTING (187 sequences)

SEQ ID NO: 1 - DNA, 4272 bp, Streptococcus pyogenes
  source 1..4272: mol_type = genomic DNA
atggactataaggaccacgacggagactacaaggatcatgatattgattacaaagacgatgacgataagatggccccaaagaagaagcggaaggtcggtatccacggagtcccagcagccgacaagaagtacagcatcggcctggacatcggcaccaactctgtgggctgggccgtgatcaccgacgagtacaaggtgcccagcaagaaattcaaggtgctgggcaacaccgaccggcacagcatcaagaagaacctgatcggagccctgctgttcgacagcggcgaaacagccgaggccacccggctgaagagaaccgccagaagaagatacaccagacggaagaaccggatctgctatctgcaagagatcttcagcaacgagatggccaaggtggacgacagcttcttccacagactggaagagtccttcctggtggaagaggataagaagcacgagcggcaccccatcttcggcaacatcgtggacgaggtggcctaccacgagaagtaccccaccatctaccacctgagaaagaaactggtggacagcaccgacaaggccgacctgcggctgatctatctggccctggcccacatgatcaagttccggggccacttcctgatcgagggcgacctgaaccccgacaacagcgacgtggacaagctgttcatccagctggtgcagacctacaaccagctgttcgaggaaaaccccatcaacgccagcggcgtggacgccaaggccatcctgtctgccagactgagcaagagcagacggctggaaaatctgatcgcccagctgcccggcgagaagaagaatggcctgttcggaaacctgattgccctgagcctgggcctgacccccaacttcaagagcaacttcgacctggccgaggatgccaaactgcagctgagcaaggacacctacgacgacgacctggacaacctgctggcccagatcggcgaccagtacgccgacctgtttctggccgccaagaacctgtccgacgccatcctgctgagcgacatcctgagagtgaacaccgagatcaccaaggcccccctgagcgcctctatgatcaagagatacgacgagcaccaccaggacctgaccctgctgaaagctctcgtgcggcagcagctgcctgagaagtacaaagagattttcttcgaccagagcaagaacggctacgccggctacattgacggcggagccagccaggaagagttctacaagttcatcaagcccatcctggaaaagatggacggcaccgaggaactgctcgtgaagctgaacagagaggacctgctgcggaagcagcggaccttcgacaacggcagcatcccccaccagatccacctgggagagctgcacgccattctgcggcggcaggaagatttttacccattcctgaaggacaaccgggaaaagatcgagaagatcctgaccttccgcatcccctactacgtgggccctctggccaggggaaacagcagattcgcctggatgaccagaaagagcgaggaaaccatcaccccctggaacttcgaggaagtggtggacaagggcgcttccgcccagagcttcatcgagcggatgaccaacttcgataagaacctgcccaacgagaaggtgctgcccaagcacagcctgctgtacgagtacttcaccgtgtataacgagctgaccaaagtgaaatacgtgaccgagggaatgagaaagcccgccttcctgagcggcgagcagaaaaaggccatcgtggacctgctgttcaagaccaaccggaaagtgaccgtgaagcagctgaaagaggactacttcaagaaaatcgagtgcttcgactccgtggaaatctccggcgtggaagatcggttcaacgcctccctgggcacataccacgatctgctgaaaattatcaaggacaaggacttcctggacaatgaggaaaacgaggacattctggaagatatcgtgctgaccctgacactgtttgaggacagagagatgatcgaggaacggctgaaaacctatgcccacctgttcgacgacaaagtgatgaagcagctgaagcggcggagatacaccggctggggcaggctgagccggaagctgatcaacggcatccgggacaagcagtccggcaagacaatcctggatttcctgaagtccgacggcttcgccaacagaaacttcatgcagctgatccacgacgacagcctgacctttaaagaggacatccagaaagcccaggtgtccggccagggcgatagcctgcacgagcacattgccaatctggccggcagccccgccattaagaagggcatcctgcagacagtgaaggtggtggacgagctcgtgaaagtgatgggccggcacaagcccgagaacatcgtgatcgaaatggccagagagaaccagaccacccagaagggacagaagaacagccgcgagagaatgaagcggatcgaagagggcatcaaagagctgggcagccagatcctgaaagaacaccccgtggaaaacacccagctgcagaacgagaagctgtacctgtactacctgcagaatgggcgggatatgtacgtggaccaggaactggacatcaaccggctgtccgactacgatgtggaccatatcgtgcctcagagctttctgaaggacgactccatcgacaacaaggtgctgaccagaagcgacaagaaccggggcaagagcgacaacgtgccctccgaagaggtcgtgaagaagatgaagaactactggcggcagctgctgaacgccaagctgattacccagagaaagttcgacaatctgaccaaggccgagagaggcggcctgagcgaactggataaggccggcttcatcaagagacagctggtggaaacccggcagatcacaaagcacgtggcacagatcctggactcccggatgaacactaagtacgacgagaatgacaagctgatccgggaagtgaaagtgatcaccctgaagtccaagctggtgtccgatttccggaaggatttccagttttacaaagtgcgcgagatcaacaactaccaccacgcccacgacgcctacctgaacgccgtcgtgggaaccgccctgatcaaaaagtaccctaagctggaaagcgagttcgtgtacggcgactacaaggtgtacgacgtgcggaagatgatcgccaagagcgagcaggaaatcggcaaggctaccgccaagtacttcttctacagcaacatcatgaactttttcaagaccgagattaccctggccaacggcgagatccggaagcggcctctgatcgagacaaacggcgaaaccggggagatcgtgtgggataagggccgggattttgccaccgtgcggaaagtgctgagcatgccccaagtgaatatcgtgaaaaagaccgaggtgcagacaggcggcttcagcaaagagtctatcctgcccaagaggaacagcgataagctgatcgccagaaagaaggactgggaccctaagaagtacggcggcttcgacagccccaccgtggcctattctgtgctggtggtggccaaagtggaaaagggcaagtccaagaaactgaagagtgtgaaagagctgctggggatcaccatcatggaaagaagcagcttcgagaagaatcccatcgactttctggaagccaagggctacaaagaagtgaaaaaggacctgatcatcaagctgcctaagtactccctgttcgagctggaaaacggccggaagagaatgctggcctctgccggcgaactgcagaagggaaacgaactggccctgccctccaaatatgtgaacttcctgtacctggccagccactatgagaagctgaagggctcccccgaggataatgagcagaaacagctgtttgtggaacagcacaagcactacctggacgagatcatcgagcagatcagcgagttctccaagagagtgatcctggccgacgctaatctggacaaagtgctgtccgcctacaacaagcaccgggataagcccatcagagagcaggccgagaatatcatccacctgtttaccctgaccaatctgggagcccctgccgccttcaagtactttgacaccaccatcgaccggaagaggtacaccagcaccaaagaggtgctggacgccaccctgatccaccagagcatcaccggcctgtacgagacacggatcgacctgtctcagctgggaggcgacaaaaggccggcggccacgaaaaaggccggccaggcaaaaaagaaaaagtaa

SEQ ID NO: 2 - DNA, 4950 bp, Francisella novicida
  source 1..4950: mol_type = genomic DNA
atgtacccatacgatgttccagattacgcttcgccgaagaaaaagcgcaaggtcgaagcgtccaattttaagatcctgcctatcgcaatcgacctgggcgtcaagaatactggcgtgtttagtgctttttatcagaaggggacctcactggagagactggacaataagaacggaaaagtgtatgaactgtccaaggattcttacactctgctgatgaacaataggaccgcacggagacaccagaggcgaggaattgacaggaaacagctggtgaagcgcctgttcaaactgatctggacagagcagctgaacctggaatgggataaggacactcagcaggccatcagcttcctgtttaatcgacggggattctcttttattactgacggctatagtcctgagtacctgaacatcgtgccagaacaggtcaaggcaatcctgatggacattttcgacgattataatggcgaggacgatctggattcctacctgaaactggccacagagcaagagagtaagatcagcgaaatctacaacaagctgatgcagaagatcctggagttcaagctgatgaaactgtgcaccgacatcaaggacgataaagtgagtaccaagacactgaaagagatcacaagctacgagttcgaactgctggccgattatctggctaactacagcgaatccctgaagacccagaaattttcctacacagacaagcagggcaatctgaaagagctgtcttactaccaccatgataagtacaacatccaggagttcctgaagagacacgccaccatcaatgacaggattctggatacactgctgactgacgatctggacatctggaacttcaacttcgagaagttcgatttcgacaagaacgaggaaaaactgcagaatcaggaagataaggaccacattcaggctcatctgcaccatttcgtgtttgcagtcaataagatcaaaagcgagatggcatccggcgggcgccatcgaagccagtacttccaggaaatcaccaacgtgctggacgagaacaatcaccaggaaggctacctgaaaaacttctgtgagaatctgcataacaagaagtacagcaatctgtccgtgaagaatctggtcaacctgattggaaatctgtccaacctggaactgaagcccctgcgcaaatacttcaacgacaagatccacgctaaagcagaccattgggatgagcagaagtttactgaaacctattgccactggattctgggcgagtggcgggtgggggtcaaggatcaggacaagaaagacggcgcaaagtattcttacaaggacctgtgtaacgagctgaagcagaaagtgactaaggccgggctggtggacttcctgctggagctggacccctgccgaaccattccaccttacctggacaacaataacagaaagccacccaaatgtcagagcctgatcctgaatcccaagtttctggataatcagtatcctaactggcagcagtacctgcaggagctgaagaaactgcagtcaatccagaactacctggacagcttcgaaaccgatctgaaggtgctgaaaagctccaaggaccagccttacttcgtcgagtacaagtctagtaaccagcagatcgcttccggccagcgggattacaaggatctggacgcaagaatcctgcagttcatttttgacagggtgaaggcctctgatgagctgctgctgaacgaaatctatttccaggcaaagaaactgaagcagaaagcctcaagcgagctggaaaagctggagtcctctaagaaactggacgaagtgatcgctaactctcagctgagtcagattctgaagtctcagcacacaaatggaatcttcgagcagggcacttttctgcatctggtgtgcaaatactataagcagcgacagagagccagggacagccgcctgtacatcatgcctgaatatcgatacgataagaaactgcacaagtacaacaacaccggccgctttgacgatgacaaccagctgctgacatattgtaatcataagccccggcagaaaagataccagctgctgaacgacctggcaggagtgctgcaggtctctcctaattttctgaaggataaaatcgggtccgatgacgatctgttcatttctaagtggctggtggagcacatccggggctttaagaaggcctgcgaagacagcctgaaaatccagaaggataacaggggactgctgaatcataagatcaacattgcacgcaataccaagggcaaatgcgagaaagaaatcttcaacctgatctgtaagattgaggggagcgaagacaagaaagggaattataagcacggactggcctacgagctgggagtgctgctgttcggagagccaaacgaggccagcaagcccgaatttgataggaaaatcaagaaattcaattcaatctacagctttgcccagatccagcagattgcctttgctgagaggaaggggaatgcaaacacatgcgccgtgtgtagtgcagacaacgcccatcgcatgcagcagatcaaaattactgagccagtcgaagacaataaggataaaatcattctgtcagcaaaggcacagcgactgcctgcaatcccaacccgaattgtggatggagctgtcaagaaaatggctacaattctggcaaagaatatcgtggacgataattggcagaacattaagcaggtcctgagcgcaaaacaccagctgcatatcccaatcattaccgagtccaacgccttcgagtttgaacccgctctggcagacgtgaagggcaaatctctgaaggatagaaggaagaaagccctggagcgaattagtcccgaaaacatcttcaaggataagaacaacagaatcaaggagtttgctaaggggatttccgcctactctggagctaacctgacagatggggacttcgatggagcaaaggaggaactggatcacatcattcctcgcagccataagaaatatggcactctgaacgacgaggctaatctgatttgcgtgacccggggcgataataagaacaaagggaaccggatcttctgtctgagagacctggccgataattacaagctgaaacagtttgagaccacagacgatctggagatcgaaaagaaaattgccgacaccatctgggatgctaataagaaggacttcaagttcggaaactatcggagcttcatcaatctgacacctcaggagcagaaagcattcagacacgccctgtttctggctgatgaaaacccaatcaagcaggcagtgatcagagccattaataaccgcaaccgaaccttcgtgaatggcacacagaggtattttgctgaggtcctggcaaataacatctacctgcgcgccaagaaagaaaatctgaacactgacaagatcagcttcgattactttggaatccctaccattggaaacggccgagggatcgctgagattcggcagctgtatgaaaaggtggacagtgatatccaggcctacgctaaaggcgacaagccacaggcctcttatagtcacctgattgatgctatgctggcattctgcatcgccgctgacgagcatcggaacgatggatctattggcctggaaatcgacaaaaactatagtctgtaccctctggataagaatactggcgaggtgttcaccaaagacatcttttcacagatcaagattaccgacaacgagttcagcgataagaaactggtcagaaagaaagctattgaagggtttaacacacacagacagatgactagggatggaatctatgcagagaattacctgcctatcctgattcataaggagctgaacgaagtgaggaaggggtacacatggaaaaattccgaggaaatcaaaattttcaagggaaagaaatacgacatccagcagctgaataacctggtgtattgtctgaagtttgtggacaaaccaatcagtattgatatccagatttcaaccctggaggaactgagaaacatcctgactaccaataacattgcagccactgccgagtactattacattaatctgaaaacccagaagctgcacgagtattacatcgaaaattacaacacagccctggggtataagaaatacagcaaggagatggagttcctgaggtccctggcttataggtctgagcgcgtgaagatcaaaagtattgacgatgtcaagcaggtcctggacaaggattcaaacttcatcatcggaaagatcacactgcccttcaagaaagagtggcagcgactgtaccgggaatggcagaacacaactatcaaagacgattatgagtttctgaagagcttctttaatgtgaagtccattactaaactgcacaagaaagtccggaaagacttctctctgcccatcagtacaaacgagggcaagtttctggtgaagagaaaaacttgggataataacttcatctaccagattctgaatgactcagatagcagggcagacgggactaaacccttcattcctgcctttgatatcagcaagaacgagattgtggaagccatcattgacagtttcacctcaaaaaacatcttttggctgccaaagaatattgagctgcagaaggtggacaacaagaacatcttcgccattgataccagcaagtggtttgaggtcgaaacaccatccgacctgcgcgatatcggcattgctaccattcagtacaagatcgacaataactcacgccccaaggtgcgagtcaaactggattacgtgatcgacgatgacagcaagattaactatttcatgaatcactcactgctgaagagccggtatcccgacaaagtcctggagatcctgaagcagagcacaatcattgagttcgaaagttcagggtttaacaaaactattaaggagatgctgggaatgaagctggccggcatctacaatgaaacctccaataactaa

SEQ ID NO: 3 - protein, 1423 aa, Streptococcus pyogenes
MDYKDHDGDYKDHDIDYKDDDDKMAPKKKRKVGIHGVPAADKKYSIGLDIGTNSVGWAVITDEYKVPSKKFKVLGNTDRHSIKKNLIGALLFDSGETAEATRLKRTARRRYTRRKNRICYLQEIFSNEMAKVDDSFFHRLEESFLVEEDKKHERHPIFGNIVDEVAYHEKYPTIYHLRKKLVDSTDKADLRLIYLALAHMIKFRGHFLIEGDLNPDNSDVDKLFIQLVQTYNQLFEENPINASGVDAKAILSARLSKSRRLENLIAQLPGEKKNGLFGNLIALSLGLTPNFKSNFDLAEDAKLQLSKDTYDDDLDNLLAQIGDQYADLFLAAKNLSDAILLSDILRVNTEITKAPLSASMIKRYDEHHQDLTLLKALVRQQLPEKYKEIFFDQSKNGYAGYIDGGASQEEFYKFIKPILEKMDGTEELLVKLNREDLLRKQRTFDNGSIPHQIHLGELHAILRRQEDFYPFLKDNREKIEKILTFRIPYYVGPLARGNSRFAWMTRKSEETITPWNFEEVVDKGASAQSFIERMTNFDKNLPNEKVLPKHSLLYEYFTVYNELTKVKYVTEGMRKPAFLSGEQKKAIVDLLFKTNRKVTVKQLKEDYFKKIECFDSVEISGVEDRFNASLGTYHDLLKIIKDKDFLDNEENEDILEDIVLTLTLFEDREMIEERLKTYAHLFDDKVMKQLKRRRYTGWGRLSRKLINGIRDKQSGKTILDFLKSDGFANRNFMQLIHDDSLTFKEDIQKAQVSGQGDSLHEHIANLAGSPAIKKGILQTVKVVDELVKVMGRHKPENIVIEMARENQTTQKGQKNSRERMKRIEEGIKELGSQILKEHPVENTQLQNEKLYLYYLQNGRDMYVDQELDINRLSDYDVDHIVPQSFLKDDSIDNKVLTRSDKNRGKSDNVPSEEVVKKMKNYWRQLLNAKLITQRKFDNLTKAERGGLSELDKAGFIKRQLVETRQITKHVAQILDSRMNTKYDENDKLIREVKVITLKSKLVSDFRKDFQFYKVREINNYHHAHDAYLNAVVGTALIKKYPKLESEFVYGDYKVYDVRKMIAKSEQEIGKATAKYFFYSNIMNFFKTEITLANGEIRKRPLIETNGETGEIVWDKGRDFATVRKVLSMPQVNIVKKTEVQTGGFSKESILPKRNSDKLIARKKDWDPKKYGGFDSPTVAYSVLVVAKVEKGKSKKLKSVKELLGITIMERSSFEKNPIDFLEAKGYKEVKKDLIIKLPKYSLFELENGRKRMLASAGELQKGNELALPSKYVNFLYLASHYEKLKGSPEDNEQKQLFVEQHKHYLDEIIEQISEFSKRVILADANLDKVLSAYNKHRDKPIREQAENIIHLFTLTNLGAPAAFKYFDTTIDRKRYTSTKEVLDATLIHQSITGLYETRIDLSQLGGDKRPAATKKAGQAKKKK

SEQ ID NO: 4 - protein, 1649 aa, Francisella novicida
MYPYDVPDYASPKKKRKVEASNFKILPIAIDLGVKNTGVFSAFYQKGTSLERLDNKNGKVYELSKDSYTLLMNNRTARRHQRRGIDRKQLVKRLFKLIWTEQLNLEWDKDTQQAISFLFNRRGFSFITDGYSPEYLNIVPEQVKAILMDIFDDYNGEDDLDSYLKLATEQESKISEIYNKLMQKILEFKLMKLCTDIKDDKVSTKTLKEITSYEFELLADYLANYSESLKTQKFSYTDKQGNLKELSYYHHDKYNIQEFLKRHATINDRILDTLLTDDLDIWNFNFEKFDFDKNEEKLQNQEDKDHIQAHLHHFVFAVNKIKSEMASGGRHRSQYFQEITNVLDENNHQEGYLKNFCENLHNKKYSNLSVKNLVNLIGNLSNLELKPLRKYFNDKIHAKADHWDEQKFTETYCHWILGEWRVGVKDQDKKDGAKYSYKDLCNELKQKVTKAGLVDFLLELDPCRTIPPYLDNNNRKPPKCQSLILNPKFLDNQYPNWQQYLQELKKLQSIQNYLDSFETDLKVLKSSKDQPYFVEYKSSNQQIASGQRDYKDLDARILQFIFDRVKASDELLLNEIYFQAKKLKQKASSELEKLESSKKLDEVIANSQLSQILKSQHTNGIFEQGTFLHLVCKYYKQRQRARDSRLYIMPEYRYDKKLHKYNNTGRFDDDNQLLTYCNHKPRQKRYQLLNDLAGVLQVSPNFLKDKIGSDDDLFISKWLVEHIRGFKKACEDSLKIQKDNRGLLNHKINIARNTKGKCEKEIFNLICKIEGSEDKKGNYKHGLAYELGVLLFGEPNEASKPEFDRKIKKFNSIYSFAQIQQIAFAERKGNANTCAVCSADNAHRMQQIKITEPVEDNKDKIILSAKAQRLPAIPTRIVDGAVKKMATILAKNIVDDNWQNIKQVLSAKHQLHIPIITESNAFEFEPALADVKGKSLKDRRKKALERISPENIFKDKNNRIKEFAKGISAYSGANLTDGDFDGAKEELDHIIPRSHKKYGTLNDEANLICVTRGDNKNKGNRIFCLRDLADNYKLKQFETTDDLEIEKKIADTIWDANKKDFKFGNYRSFINLTPQEQKAFRHALFLADENPIKQAVIRAINNRNRTFVNGTQRYFAEVLANNIYLRAKKENLNTDKISFDYFGIPTIGNGRGIAEIRQLYEKVDSDIQAYAKGDKPQASYSHLIDAMLAFCIAADEHRNDGSIGLEIDKNYSLYPLDKNTGEVFTKDIFSQIKITDNEFSDKKLVRKKAIEGFNTHRQMTRDGIYAENYLPILIHKELNEVRKGYTWKNSEEIKIFKGKKYDIQQLNNLVYCLKFVDKPISIDIQISTLEELRNILTTNNIAATAEYYYINLKTQKLHEYYIENYNTALGYKKYSKEMEFLRSLAYRSERVKIKSIDDVKQVLDKDSNFIIGKITLPFKKEWQRLYREWQNTTIKDDYEFLKSFFNVKSITKLHKKVRKDFSLPISTNEGKFLVKRKTWDNNFIYQILNDSDSRADGTKPFIPAFDISKNEIVEAIIDSFTSKNIFWLPKNIELQKVDNKNIFAIDTSKWFEVETPSDLRDIGIATIQYKIDNNSRPKVRVKLDYVIDDDSKINYFMNHSLLKSRYPDKVLEILKQSTIIEFESSGFNKTIKEMLGMKLAGIYNETSNN

SEQ ID NO: 5 - DNA, 5133 bp, unidentified
  misc_feature 1..5133: note = source = /note="Description of Unknown: BE3 sequence"
  source 1..5133: mol_type = genomic DNA
atgagctcagagactggcccagtggctgtggaccccacattgagacggcggatcgagccccatgagtttgaggtattcttcgatccgagagagctccgcaaggagacctgcctgctttacgaaattaattgggggggccggcactccatttggcgacatacatcacagaacactaacaagcacgtcgaagtcaacttcatcgagaagttcacgacagaaagatatttctgtccgaacacaaggtgcagcattacctggtttctcagctggagcccatgcggcgaatgtagtagggccatcactgaattcctgtcaaggtatccccacgtcactctgtttatttacatcgcaaggctgtaccaccacgctgacccccgcaatcgacaaggcctgcgggatttgatctcttcaggtgtgactatccaaattatgactgagcaggagtcaggatactgctggagaaactttgtgaattatagcccgagtaatgaagcccactggcctaggtatccccatctgtgggtacgactgtacgttcttgaactgtactgcatcatactgggcctgcctccttgtctcaacattctgagaaggaagcagccacagctgacattctttaccatcgctcttcagtcttgtcattaccagcgactgcccccacacattctctgggccaccgggttgaaaagcggcagcgagactcccgggacctcagagtccgccacacccgaaagtgataaaaagtattctattggtttagccatcggcactaattccgttggatgggctgtcataaccgatgaatacaaagtaccttcaaagaaatttaaggtgttggggaacacagaccgtcattcgattaaaaagaatcttatcggtgccctcctattcgatagtggcgaaacggcagaggcgactcgcctgaaacgaaccgctcggagaaggtatacacgtcgcaagaaccgaatatgttacttacaagaaatttttagcaatgagatggccaaagttgacgattctttctttcaccgtttggaagagtccttccttgtcgaagaggacaagaaacatgaacggcaccccatctttggaaacatagtagatgaggtggcatatcatgaaaagtacccaacgatttatcacctcagaaaaaagctagttgactcaactgataaagcggacctgaggttaatctacttggctcttgcccatatgataaagttccgtgggcactttctcattgagggtgatctaaatccggacaactcggatgtcgacaaactgttcatccagttagtacaaacctataatcagttgtttgaagagaaccctataaatgcaagtggcgtggatgcgaaggctattcttagcgcccgcctctctaaatcccgacggctagaaaacctgatcgcacaattacccggagagaagaaaaatgggttgttcggtaaccttatagcgctctcactaggcctgacaccaaattttaagtcgaacttcgacttagctgaagatgccaaattgcagcttagtaaggacacgtacgatgacgatctcgacaatctactggcacaaattggagatcagtatgcggacttatttttggctgccaaaaaccttagcgatgcaatcctcctatctgacatactgagagttaatactgagattaccaaggcgccgttatccgcttcaatgatcaaaaggtacgatgaacatcaccaagacttgacacttctcaaggccctagtccgtcagcaactgcctgagaaatataaggaaatattctttgatcagtcgaaaaacgggtacgcaggttatattgacggcggagcgagtcaagaggaattctacaagtttatcaaacccatattagagaagatggatgggacggaagagttgcttgtaaaactcaatcgcgaagatctactgcgaaagcagcggactttcgacaacggtagcattccacatcaaatccacttaggcgaattgcatgctatacttagaaggcaggaggatttttatccgttcctcaaagacaatcgtgaaaagattgagaaaatcctaacctttcgcataccttactatgtgggacccctggcccgagggaactctcggttcgcatggatgacaagaaagtccgaagaaacgattactccatggaattttgaggaagttgtcgataaaggtgcgtcagctcaatcgttcatcgagaggatgaccaactttgacaagaatttaccgaacgaaaaagtattgcctaagcacagtttactttacgagtatttcacagtgtacaatgaactcacgaaagttaagtatgtcactgagggcatgcgtaaacccgcctttctaagcggagaacagaagaaagcaatagtagatctgttattcaagaccaaccgcaaagtgacagttaagcaattgaaagaggactactttaagaaaattgaatgcttcgattctgtcgagatctccggggtagaagatcgatttaatgcgtcacttggtacgtatcatgacctcctaaagataattaaagataaggacttcctggataacgaagagaatgaagatatcttagaagatatagtgttgactcttaccctctttgaagatcgggaaatgattgaggaaagactaaaaacatacgctcacctgttcgacgataaggttatgaaacagttaaagaggcgtcgctatacgggctggggacgattgtcgcggaaacttatcaacgggataagagacaagcaaagtggtaaaactattctcgattttctaaagagcgacggcttcgccaataggaactttatgcagctgatccatgatgactctttaaccttcaaagaggatatacaaaaggcacaggtttccggacaaggggactcattgcacgaacatattgcgaatcttgctggttcgccagccatcaaaaagggcatactccagacagtcaaagtagtggatgagctagttaaggtcatgggacgtcacaaaccggaaaacattgtaatcgagatggcacgcgaaaatcaaacgactcagaaggggcaaaaaaacagtcgagagcggatgaagagaatagaagagggtattaaagaactgggcagccagatcttaaaggagcatcctgtggaaaatacccaattgcagaacgagaaactttacctctattacctacaaaatggaagggacatgtatgttgatcaggaactggacataaaccgtttatctgattacgacgtcgatcacattgtaccccaatcctttttgaaggacgattcaatcgacaataaagtgcttacacgctcggataagaaccgagggaaaagtgacaatgttccaagcgaggaagtcgtaaagaaaatgaagaactattggcggcagctcctaaatgcgaaactgataacgcaaagaaagttcgataacttaactaaagctgagaggggtggcttgtctgaacttgacaaggccggatttattaaacgtcagctcgtggaaacccgccaaatcacaaagcatgttgcacagatactagattcccgaatgaatacgaaatacgacgagaacgataagctgattcgggaagtcaaagtaatcactttaaagtcaaaattggtgtcggacttcagaaaggattttcaattctataaagttagggagataaataactaccaccatgcgcacgacgcttatcttaatgccgtcgtagggaccgcactcattaagaaatacccgaagctagaaagtgagtttgtgtatggtgattacaaagtttatgacgtccgtaagatgatcgcgaaaagcgaacaggagataggcaaggctacagccaaatacttcttttattctaacattatgaatttctttaagacggaaatcactctggcaaacggagagatacgcaaacgacctttaattgaaaccaatggggagacaggtgaaatcgtatgggataagggccgggacttcgcgacggtgagaaaagttttgtccatgccccaagtcaacatagtaaagaaaactgaggtgcagaccggagggttttcaaaggaatcgattcttccaaaaaggaatagtgataagctcatcgctcgtaaaaaggactgggacccgaaaaagtacggtggcttcgatagccctacagttgcctattctgtcctagtagtggcaaaagttgagaagggaaaatccaagaaactgaagtcagtcaaagaattattggggataacgattatggagcgctcgtcttttgaaaagaaccccatcgacttccttgaggcgaaaggttacaaggaagtaaaaaaggatctcataattaaactaccaaagtatagtctgtttgagttagaaaatggccgaaaacggatgttggctagcgccggagagcttcaaaaggggaacgaactcgcactaccgtctaaatacgtgaatttcctgtatttagcgtcccattacgagaagttgaaaggttcacctgaagataacgaacagaagcaactttttgttgagcagcacaaacattatctcgacgaaatcatagagcaaatttcggaattcagtaagagagtcatcctagctgatgccaatctggacaaagtattaagcgcatacaacaagcacagggataaacccatacgtgagcaggcggaaaatattatccatttgtttactcttaccaacctcggcgctccagccgcattcaagtattttgacacaacgatagatcgcaaacgatacacttctaccaaggaggtgctagacgcgacactgattcaccaatccatcacgggattatatgaaactcggatagatttgtcacagcttgggggtgactctggtggttctactaatctgtcagatattattgaaaaggagaccggtaagcaactggttatccaggaatccatcctcatgctcccagaggaggtggaagaagtcattgggaacaagccggaaagcgatatactcgtgcacaccgcctacgacgagagcaccgacgagaatgtcatgcttctgactagcgacgcccctgaatacaagccttgggctctggtcatacaggatagcaacggtgagaacaagattaagatgctctctggtggttctcccaagaagaagaggaaagtctaa

SEQ ID NO: 6 - protein, 1710 aa, unidentified
  REGION 1..1710: note = source = /note="Description of Unknown: BE3 sequence"
MSSETGPVAVDPTLRRRIEPHEFEVFFDPRELRKETCLLYEINWGGRHSIWRHTSQNTNKHVEVNFIEKFTTERYFCPNTRCSITWFLSWSPCGECSRAITEFLSRYPHVTLFIYIARLYHHADPRNRQGLRDLISSGVTIQIMTEQESGYCWRNFVNYSPSNEAHWPRYPHLWVRLYVLELYCIILGLPPCLNILRRKQPQLTFFTIALQSCHYQRLPPHILWATGLKSGSETPGTSESATPESDKKYSIGLAIGTNSVGWAVITDEYKVPSKKFKVLGNTDRHSIKKNLIGALLFDSGETAEATRLKRTARRRYTRRKNRICYLQEIFSNEMAKVDDSFFHRLEESFLVEEDKKHERHPIFGNIVDEVAYHEKYPTIYHLRKKLVDSTDKADLRLIYLALAHMIKFRGHFLIEGDLNPDNSDVDKLFIQLVQTYNQLFEENPINASGVDAKAILSARLSKSRRLENLIAQLPGEKKNGLFGNLIALSLGLTPNFKSNFDLAEDAKLQLSKDTYDDDLDNLLAQIGDQYADLFLAAKNLSDAILLSDILRVNTEITKAPLSASMIKRYDEHHQDLTLLKALVRQQLPEKYKEIFFDQSKNGYAGYIDGGASQEEFYKFIKPILEKMDGTEELLVKLNREDLLRKQRTFDNGSIPHQIHLGELHAILRRQEDFYPFLKDNREKIEKILTFRIPYYVGPLARGNSRFAWMTRKSEETITPWNFEEVVDKGASAQSFIERMTNFDKNLPNEKVLPKHSLLYEYFTVYNELTKVKYVTEGMRKPAFLSGEQKKAIVDLLFKTNRKVTVKQLKEDYFKKIECFDSVEISGVEDRFNASLGTYHDLLKIIKDKDFLDNEENEDILEDIVLTLTLFEDREMIEERLKTYAHLFDDKVMKQLKRRRYTGWGRLSRKLINGIRDKQSGKTILDFLKSDGFANRNFMQLIHDDSLTFKEDIQKAQVSGQGDSLHEHIANLAGSPAIKKGILQTVKVVDELVKVMGRHKPENIVIEMARENQTTQKGQKNSRERMKRIEEGIKELGSQILKEHPVENTQLQNEKLYLYYLQNGRDMYVDQELDINRLSDYDVDHIVPQSFLKDDSIDNKVLTRSDKNRGKSDNVPSEEVVKKMKNYWRQLLNAKLITQRKFDNLTKAERGGLSELDKAGFIKRQLVETRQITKHVAQILDSRMNTKYDENDKLIREVKVITLKSKLVSDFRKDFQFYKVREINNYHHAHDAYLNAVVGTALIKKYPKLESEFVYGDYKVYDVRKMIAKSEQEIGKATAKYFFYSNIMNFFKTEITLANGEIRKRPLIETNGETGEIVWDKGRDFATVRKVLSMPQVNIVKKTEVQTGGFSKESILPKRNSDKLIARKKDWDPKKYGGFDSPTVAYSVLVVAKVEKGKSKKLKSVKELLGITIMERSSFEKNPIDFLEAKGYKEVKKDLIIKLPKYSLFELENGRKRMLASAGELQKGNELALPSKYVNFLYLASHYEKLKGSPEDNEQKQLFVEQHKHYLDEIIEQISEFSKRVILADANLDKVLSAYNKHRDKPIREQAENIIHLFTLTNLGAPAAFKYFDTTIDRKRYTSTKEVLDATLIHQSITGLYETRIDLSQLGGDSGGSTNLSDIIEKETGKQLVIQESILMLPEEVEEVIGNKPESDILVHTAYDESTDENVMLLTSDAPEYKPWALVIQDSNGENKIKMLSGGSPKKKRKV

SEQ ID NO: 7 - DNA, 13761 bp, unidentified
  misc_feature 1..13761: note = source = /note="Description of Unknown: HB-EGF sequence"
  source 1..13761: mol_type = genomic DNA
attcggccgaaggagctacgcgggccacgctgctggctggcctgacctaggcgcgcggggtcgggcggccgcgcgggcgggctgagtgagcaagacaagacactcaagaagagcgagctgcgcctgggtcccggccaggcttgcacgcagaggcgggcggcagacggtgcccggcggaatctcctgagctccgccgcccagctctggtgccagcgcccagtggccgccgcttcgaaagtgactggtgcctcgccgcctcctctcggtgcgggaccatgaagctgctgccgtcggtggtgctgaagctctttctggctgcaggtaagagggctgccgacgcccccggagatcggggggatgggggcgttgtgctgggggcatgggggaaggtcgccgcagcgcacccggcacgggccacttggtggggcccttgcgctctggcggacgggcgtcggcatcggtgcgtgttggtcaggggtctgggcgggtgtctgatgcggcctggcctctcgcccgcagttctctcggcactggtgactggcgagagcctggagcggcttcggagagggctagctgctggaaccagcaacccggaccctcccactgtatccacggaccagctgctacccctaggaggcggccgggaccggaaagtccgtgacttgcaagaggcagatctggaccttttgagaggtgggtgtggaggccccccatccttggaccttggtgggctgttgaagaataagcagatccaagattcttgctgtttgggcaatactgtgggttgagggtattcatggagaacctcggggaaaagctgatcggcctgatgggcactgggggatcctggaatataggtcccactctctctctcttgtcattgcctcacctgctgggttgctgcccttctgggtactccggggcaaattgaatcagacgtgttgtctggggttgttacgttcttcttaggtaagctgggtgataggaacaaggaatggttgagatgctttccctagagctactatgtaaaaatgggcgccagttctaattcccatatcaaatgactattatatataaaatagaggtaacacatgcggagatgcccaggcacatctctagaaagtgtgcagtgttggcctcctccatccacctgtctccagattggggaaacagaggggaatgaggagctcttggccgccctagatgaggctgtgaatggtgagcactgagcccctagggggctgtattaaaatgctggatatctgtgaatgctaccggaaacctgcagcttactgagcaccttgcattcctgaggagactccaaatggggagggctgtgtaggatcctccaaccagcctctttggctgtggccaagtacaggtacagggcagagtccagagcctgccagctctcctgcctccaaacctgaggagattatccagagtagagcaaggactcagcactgtaccctggaatgactatatttggttggacagatgcccacctgttctagttccacctgctcctcagctgcccttctccctcattcccaggagctttccttggatactctctctactttgtataaatcaagcacatactccaaaactgagcctgggctcccatacttcatcctctcccagtggccctctggggttgcccatgacctgaacagcctggattctcctggccctctcctcctaggctgggcagggctgggctgtgactcaccccacccccaccccccacccacacggctgctcctcttacctctgcagacctgactcactgctccctgtccatggcaggagcctggctgtcaccctgcaccttctccctcccctttctgattggcttggcccccctgccttgctctccccgaagctctggtcactgggttcctctgaccacctgtatcaccttctgagctctgagggggcctgggactggatgagaggaaatgaaagactgtgggggctgctggcacctacttctcttcccttcttttggctttgctgggcaaggactatttttcaggtctggggatcctaccacctaaaataaatgactgctaccatttattaaattcctactgtgttctaggcacttgatatgttatcctggctaatgtaacacttatagcaaccttttgagatagttactttggctatccacattttactgagaacctgaggttcagaggagttaagtgactgcccacagtaaatagctgaaattggagcacaggtctatggacttcagagcccattcatgcctggatcagcatctcaggtgctctagacttgtgagagggaggagatgggagtgtgtgaggcagcttggtgtggtgaggaaggacattggagtgaagtccagagaacacagttctaatcccaatcctgcatgaccttgagtaagtcactctgcctgccatgagttttttctttttttcttttttttttttttaaacatagtctcactctgtcacccaggctggagtgcaatggcacgatctcagctcactgcaatctctgcctcccaggttcaagtgattctcctgcctcagcctcctgagtagctgcgataacaggcacacaccaccacgcccggctaatttttgtattttttgtagagatgagatttttgccatgttggcaaggctggtctcgaactcccgacctcaggtgatccacctgcctcagcctcccaaagtgttgggattacaggcgtgagccaccgtgcctggccacatggtattctttgaagtccctctagcttgagactctaagtctctagtctaacgtatcatgcttacccttctgtaagacacatggctgtagccatggatgtgggcacctttttcctgatgggggataaaagggtgggattgggctgataggcatagtccctggtcaatcccagctggatatctgggtgaggctgtttttcccccagtctctctgaagcatggaaagaaggagggagtcatcattgttccagttccttctggacagttccttactttccatttttctatcccttgtacaccctgtaccccccaatccagagagctataaacaggacattgggggttaaatatgaatgaatctttgagaaagtgggtgagctgtaaagggtatgcaagttaaatattttgcttgaagttgaaaaagcaaggccgtgaccagggctggcctgcttgctgttcctgagccaggctctgccctgggctcatagtactaaggggtgccccagaagagaccacctgaacacatggacactgttcttatattaggagccctccaaccccagaacctccaagtaccttctctagaagcaatttttgtgtgtgacactgtctttctgcaagtggttcactgagtacagcatcaggaaatgaggctgattgaaggccaaaatagaatgaagtgggtgtgggggagtaggagatgggggtgtaaggtggacagtggggtggaggtgaggttggtagaattgcccagttactcaacaaaagcattctgagaatgaggctcttacacagagactgtgaaatgccttccttgggacccaccctagcttctacttcctaccgaggttccctctttctggtggttctgcccaatcttcctgctcttccttctgcctcttaggaggcactgagctaaggggccttcccagatctctgacttcaggtggaatcaaagcatatatactcctttcaagcactatgctcttctgattttcttcccaaagagtcagactttaacagagtgcttttctcctacagtcactttatcctccaagccacaagcactggccacaccaaacaaggaggagcacgggaaaagaaagaagaaaggcaaggggctagggaagaagagggacccatgtcttcggaaatacaaggacttctgcatccatggagaatgcaaatatgtgaaggagctccgggctccctcctgcatgtaagtgccccttccccagggctgaatctcatcagcacactttgtcagccacgtggctgttcctcgttgtcactgttccttgaattcataatttcacccagtttcttctcaacctctgggcggaagttgggaggaggggaaatatatttttagtcagcggaagccccctcccccctataggatgcaatttcctgtggtatggttttgtgacgtgctttaatccttggggacatttcctgcttgcccagaaatgagcatgtggctaggacagctggcacctgaaggcaggcccttaattcttgcctgatgccctactctgggagggagaagccagtaggaaacatggcagagtgggcttccagggcagagtagagctcctgtgggaaggtaggaagtgcatttggatgcatgatgtataggtatgtgtgtatttgggtttatgtgcatgtaagtgtgcaaatgtggattgactgtgaggcatggcaggactgtacagagagggatcatcatggcggcaggttgaggcctctctttcttcttccttatcccagcaaggacgaggaggtgggagacatggagagtactggcctttggccacgttgtgagagaacaattcctttgtgcagggttcacaggaaatggaacctgacccattaggcatcagcccccggtcaggcaacatcaccccttccctgggtaggtgtgtgggtggaggggctgtgggttccttagcctctctcctaagccaaacccagcaaacggctgccttggcaacccctcagggatgacagcactgccatgctctctggcaggcataatgttgccactgtgcctgaggccaacaccctgcgtcaggctgcaaacatccattcccttccctgtggggagggaggctctgggggccttagtgggagactctggacagggccaagagactgttgtatgcacactgcctccagcctgtcaagaaggcggcgtgcctggcatcccttctactggtgattggtgcagatcccttagctttttaaagcttccttgttttgtctgatcacacacagcagagctgccctgtatttggcagttggcagacagacccatcactccccaccatgtccacagtcacttgtgcatcctttcctataacatccttgtcaggagcttggtattagagggagttgtttaagagtggcatagaaagcccccatattatccttcccaaggtcttgggacagggtgggaaatgttcatcttaaatttgtaaaatggcatcattagtacagggtgaagaaggtgactcaagtagtcaaggtggattgaggtcaggaatctgtctataccagattggtcctgggcattttggtggatggatgtggggcttgcactgtgtggttgagaggccttataaggttgccctcctggagagctggactcggatgaccacctaaacccagagaacctgatatgggtgcccaggccaccttcccagtggtccctagggatagtgataactataatgatgtcatatctcctttgtcccagagtttcagtgtttatatataatatgagttgagcccaagtatgttgagcccctatttggtggcagacactactttaggagctggagagatatagtttcctgggatttttcaaaagccctctgctgagtaggcaggacttggtacctctacttgaaaggtgatgaaactggagccagaaaataggaagtaatttgcctgaggtcaatagctaaataagtagttggaaataagacagagtctcagtacctgactcctagtccaacatgcttttcatgccctcaagctgtactgggtgttggctttcatctttctttcctgtatctgtccttatagagttggagcagcattttatagagggcagagggcagctgttgtcctagaggtctcttattcttttactagtctaacagcacagcaatctgatttgaaaactttacattaacttcttgggcagaattttctttttctttgttcttttctttctttctttctttttttttttttttttttttttgagacagagtctcactctgtctcccatgctggggtgcagtggtgtgatctcagctcactgcaacctctgcctcctgggttcaagcaattctcctgcctcagcctcctaagtggctgggactacaggcacctgccaccatgccgaattaataatttttatatttttagtagagacgtagttttgccgtgttggccaggctggtcttgaactcttgacctcaggtgatccgcctgcctcagcctcccaaagtgctgggattacaggcatgagccaccatatctagccttttttttttttgagatggaatctcgctctgtcacccaggctggagtgcagtgacacaatctcggctctctgcagcctccgcctcccagattaaagtgattttcctgcttcagcctcctgagcagctggtattacaggcacatgcccccacatctggctaatttttaaatttttgtggagatggggtttcaccatgttggccaggctggtcttgaactcctaacctcaagtaatcagcctgccttggactcccaaagtgctgggattacaggcgtgggccaccacttcctgggcagattttcagggggttgattgcatgtctggactggccccctactgcctcctgcccttgctactcagggcagaaagcagcaagaagacagaaatcctggtttgggggaatgtgacatctgtgcacgttcatctggggatctttgtggctcttgtttgactccagacccaggaaccactagccagggtgtgtccaggctgctgtggtgagcctgaggctagctggcttcctaaactagccctctgcagccaccatgaacaggaaaaccctttttgtgtcaccagccaaaagttgccctcaaagagtagtttctgctgggcacagtggctcacacctgtaatcacagcactttgggaggccgaggcacgtgggtcgcctgaggtcaggagttcgagaccagcctggccaacatagagaaacccccgtctctactaaaaatacaaaaattagctgggtgttgtggcgggcgcctgtaatctcagctactagagaggctgaggcaggagaatctctcaaacccaggaggcagaacttgcagtgagccgagatagtgccattgcactccagcctaggcaacaagagcaaaactccatctcaaaaaaataataataataaataaataaaagagtagtttcctgggattcctgactagttgcctacccagaaattggctgcagagtttcctgtggctggaggaaaactggggacacttgggctgaggaggactcagagctggaggagagacaggctagggggctctacttggcctcactgcccaggtgctaagaaggaatggtgatcccgcttctcttgtctccatctgacttgggtgccccattcctcaggccatgggcagtaacctctggagtctgattatgtaataactcacacaatgtgggacttggcctttataaagccctttcatttgtattacctcattttatcttttcacaatactctagtgaagtaggcatttcttatccctgtgttttacatgaggaaaccaatgtttagaaaggtaacgtgacttgcccaaaattacctggctagaaatagcagcagaaccagtctggaactcatgcactcagtctcctccatccagacgtgtcccctccacctcctggggtaaaggtggagaaatccagtttggaagatgtctctggaccctagagggttcttgcatctgttgtaatacaagttctgaaatgggtcacagacgtgggtgggaagaatgtgtcctagtctggtgggtggctggctctggacaagacacaaaattttgcccctaccctgggatgcttggaatgtactcatcccccctccttctctggggaagccaggagttgtctgcaaagggagggggaggtaggtaatattaggatgtttacattattatccttttgactcagggtgggggtggagggattatgtaactgaattgcgggactctgaggccaaactttatttctatcttctgagtaactacctgtggagtttgaatgatggactggaagtgaaaaacagactcaacttcagcttccctcctcccaggaaagcaaagtctctgaagtcatccagactgctgttgaatcctggctctacgactcactagctttgtaaccttgggcgaggtgtttaacaaaagctaagcctcagtccatctttaaaatggggctagtaacttctccttcacagagctggctttaaatgaaataattcttgtaaagcagttagcacaaagtacttggctcatggtaagccttcaatgattgctaattattattctttattattcaagttatgagtaataaataataataacatagtcagagagaagggtcagactgccccccaggagcctatcagatatgcttccttggagttacctgcgctatcctgcattgttcaaagtggaaggaatgatgaatttggaatctgccaagacttgttcctagtcttagccctgctgcttcctagttgtgccacttttggtgaatcacttaatttctctgacccttaatcttagcttttccatctgtaatatggggttgtacctgcctaccagaatgttaggaggctcagttgagctagtagataaggctagtggcttgtgaatggtaaactgctgtgcacaagtgattttccaggggtgcttgtgcaagtgtcctctatgtcctggcaggataggggtcgcttttaggcctacatgggctgatgggacagatacatggagaggctgggcaaggaactgtggactgtgctatacgtatagtgggcctgacctacatttatcctgctgtgaggtggtttctcgaagtacccaggaggaactagggcagggagaggctcagggcaggaaagcaagaatgcagtaccacccagcctggcccctctgccactgctggttgtggacaagtctgtctcttggagcttccctggtgctctgtccgcaggaagaagggattccttgttctgaggtaccagagaaagcacctccttcccagagaaagcacagctcagaaaagagggccaccaggttcttggtgcttccttcagcagctggtggtctaaagtcctcaggcagacagtgccactgtgccccctggctggatggtaggcagttgtcaggtgtgagtgggcagcacactgagctcagagtcagacaatctacatctacatcttcatttctgtcttactgtgtgaccttgggaaaaccactccacctttctgtaaaacagggctcctacttatatcaaaggatctctgggatgctcagataaaggaaaggatgtgaatgtgcttcttcaactgtaagcacgtctgagtctttctaagagcttcaaggaaatgctttgtgttagaaaaggcagttgccagcccggtgtggtggctcatgcctgtaatccttgcacattgggaggcagaggcgggtggatcacctgaggtcaggagtttgagaccagcctagttaacatggtgaaactccgtctcttctaaaaaattacaaaaattagctgggcgtggtggcgggcacctgtaatcccagctacttgggaggctggggcaggagaatcacttgaatccggaggtaggggttgcagtgagccaagattgcgccactgcactccagcctgggagacagagcaagactctgtctcaaaaaaaaaaaaaaaaaaagaaaaagaaaaagaaaaggcagttgccatgtgatttatttcttgagtgagaagagccaagggattgtttctgacagtcttccatgctctggcagggcagctgggcagaaagatgtttcttgatttgtttggtttgtcctgtgatgaaagaggcctggtagctcagcgtgcagaggccaaaggccagagttgagctcccaagttgggccctgcacccagggggagctggagttaaatgaaggaaacttgagaaaaacgactcctggcagaggcacagggcctattaataggctggacagcagtggagagggactggacgctggaagcacgatggggaaggctgggtttatttctgggtcagaatgttgaggggcctcactggagggagtgatacgaattccctcaatttagcctaccagctcttgtgcccaagccctcataagtggcttaaacagaacgcctgaacacacatgtcataaatcagccacacgtggaacatatctagctgaggccttcaagtcctcccttgctttttccatgcctagaacaggattctcagcccagagaaccagaggaaatggaaaaggggagggtgtcaagtgagagaggaatgctacagagctttcagaggggctttaaagagttttctactagaggagaaggatggaggatgggcagggatcgtggtcagggattgacaggctgagggtatgaggaatggggtttggcttatgcaggtgggccattgccaagagaggccaaagcactaactccatctccttcttgttctgtcttgaactagctgccacccgggttaccatggagagaggtgtcatgggctgagcctcccagtggaaaatcgcttatatacctatgaccacacaaccatcctggccgtggtggctgtggtgctgtcatctgtctgtctgctggtcatcgtggggcttctcatgtttaggtgagtgttggggtcccctgcaggctgtttctgcaaatcactccctttcttcctcctcctgggccctctccttgatggtcacatgcacttccctcaatctttccaaatcatgggctagctccggggtgtagattctccaaaaacctggtatttctggcatgacatgagtcctgtgtctagagcccagggtcaaatttgcgaggccatagcaggttctgctcctcacaggagttcttttcctgcctccatgacccagctacccactcatggagtcactttgtcacacatttctttctcctggctgttctttgatggcattagtatgtggtttggtagtcaaggtgtgggtggtgctagtggtatatccttccacttctgaggcgtctggacctcaggccctgctttctaatccaggtatgctctagcttgggagacccaccaagcactctatgcctgttttctttctttctttttttttttttttttttgagacagagtcttgctctgtcgcccaggctggagtgcagtggtgtgatctcggctcactgcaaactccgcctcctgggttcacgccattctcctgcctcagcctcctgagtagctgggactacaggcacccgccaccacacccagctaattttttctattttttagtagagacggggtttcaccatgttagccaggatggtctcgatctcctgacctcgtgatctgcccgcctcggcctcccaaagtgctgggattacaggcatgagccaccgtgcctagctctatgcctgttttcaagcagtgtaactcatctgtcatgagacctggaacaagttactgtctttctgaggattgtaaccttgtagtgattgtaatgtttgtccatctacctcataaggatgttgtgaggatcacgtaaatgaggtgaaagctatttgtaaattgcatcctgctattagagacaggagttcctcggggcagttgggcctttgaccagagtttgggctgccctactgcctgggcttttccaagtagtagaggaaaccaccatggcagagttctttggaaggacctgctctggacctgcactttgtcatagcaggcagggcttattcacaaaacttatcttcctcaggtaccataggagaggaggttatgatgtggaaaatgaagagaaagtgaagttgggcatgactaattcccactgagagagacttgtgctcaaggtaacgctccatcctttgccccatgacatgattatcctttgtcccctttcctggctgtgcttcagtgggtgctgaattcttcatataggggttgggggccaggctactgtgacattaatatcccattgcagaattattttcaaaaagactcagtgcttcacttaaggtaaaagttgctagagagacacctaagagagatgcctgagaggacagcttctcccaccctcatcccctcccttcccctcccctctcctcccctgggagacagagtgaaaccctgtctcaaaaagtttaaaaataaaaaagactggaccaggaaaatcttaagacttctttagactggacctggctttacatgccttccttttgtgctttaggaatcggctggggactgctacctctgagaagacacaaggtgatttcagactgcagaggggaaagacttccatctagtcacaaagactccttcgtccccagttgccgtctaggattgggcctcccataattgctttgccaaaataccagagccttcaagtgccaaacagagtatgtccgatggtatctgggtaagaagaaagcaaaagcaagggaccttcatgcccttctgattcccctccaccaaaccccacttcccctcataagtttgtttaaacacttatcttctggattagaatgccggttaaattccatatgctccaggatctttgactgaaaaaaaaaaagaagaagaagaaggagagcaagaaggaaagatttgtgaactggaagaaagcaacaaagattgagaagccatgtactcaagtaccaccaagggatctgccattgggaccctccagtgctggatttgatgagttaactgtgaaataccacaagcctgagaactgaattttgggacttctacccagatggaaaaataacaactatttttgttgttgttgtttgtaaatgcctcttaaattatatatttattttattctatgtatgttaatttatttagtttttaacaatctaacaataatatttcaagtgcctagactgttactttggcaatttcctggccctccactcctcatccccacaatctggcttagtgccacccacctttgccacaaagctaggatggttctgtgacccatctgtagtaatttattgtctgtctacatttctgcagatcttccgtggtcagagtgccactgcgggagctctgtatggtcaggatgtaggggttaacttggtcagagccactctatgagttggacttcagtcttgcctaggcgattttgtctaccatttgtgttttgaaagcccaaggtgctgatgtcaaagtgtaacagatatcagtgtctccccgtgtcctctccctgccaagtctcagaagaggttgggcttccatgcctgtagctttcctggtccctcacccccatggccccaggcccacagcgtgggaactcactttcccttgtgtcaagacatttctctaactcctgccattcttctggtgctactccatgcaggggtcagtgcagcagaggacagtctggagaaggtattagcaaagcaaaaggctgagaaggaacagggaacattggagctgactgttcttggtaactgattacctgccaattgctaccgagaaggttggaggtggggaaggctttgtataatcccacccacctcaccaaaacgatgaagttatgctgtcatggtcctttctggaagtttctggtgccatttctgaactgttacaacttgtatttccaaacctggttcatatttatactttgcaatccaaataaagataacccttattccata

SEQ ID NO: 8 - protein, 208 aa, unidentified
  REGION 1..208: note = source = /note="Description of Unknown: HB-EGF sequence"
MKLLPSVVLKLFLAAVLSALVTGESLERLRRGLAAGTSNPDPPTVSTDQLLPLGGGRDRKVRDLQEADLDLLRVTLSSKPQALATPNKEEHGKRKKKGKGLGKKRDPCLRKYKDFCIHGECKYVKELRAPSCICHPGYHGERCHGLSLPVENRLYTYDHTTILAVVAVVLSSVCLLVIVGLLMFRYHRRGGYDVENEEKVKLGMTNSH

SEQ ID NO: 9 - DNA, 24 bp, synthetic construct
  misc_feature 1..24: note = source = /note="Description of Artificial Sequence: Synthetic primer"
  source 1..24: mol_type = other DNA
accgaatcacccaggcggtgtagt

SEQ ID NO: 10 - DNA, 24 bp, synthetic construct
  misc_feature 1..24: note = source = /note="Description of Artificial Sequence: Synthetic primer"
  source 1..24: mol_type = other DNA
aaacactacaccgcctgggtgatt

SEQ ID NO: 11 - DNA, 24 bp, synthetic construct
  misc_feature 1..24: note = source = /note="Description of Artificial Sequence: Synthetic primer"
  source 1..24: mol_type = other DNA
accgcaggttccacgggatgctct

SEQ ID NO: 12 - DNA, 24 bp, synthetic construct
  misc_feature 1..24: note = source = /note="Description of Artificial Sequence: Synthetic primer"
  source 1..24: mol_type = other DNA
aaacagagcatcccgtggaacctg

SEQ ID NO: 13 - DNA, 23 bp, synthetic construct
  misc_feature 1..23: note = source = /note="Description of Artificial Sequence: Synthetic primer"
  source 1..23: mol_type = other DNA
accggcactgcggctggaggtgg

SEQ ID NO: 14 - DNA, 23 bp, synthetic construct
  misc_feature 1..23: note = source = /note="Description of Artificial Sequence: Synthetic primer"
  source 1..23: mol_type = other DNA
aaacccacctccagccgcagtgc

SEQ ID NO: 15 - DNA, 24 bp, synthetic construct
  misc_feature 1..24: note = source = /note="Description of Artificial Sequence: Synthetic primer"
  source 1..24: mol_type = other DNA
accgcacctctctccatggtaacc

SEQ ID NO: 16 - DNA, 24 bp, synthetic construct
  misc_feature 1..24: note = source = /note="Description of Artificial Sequence: Synthetic primer"
  source 1..24: mol_type = other DNA
aaacggttaccatggagagaggtg

SEQ ID NO: 17 - DNA, 24 bp, synthetic construct
  misc_feature 1..24: note = source = /note="Description of Artificial Sequence: Synthetic primer"
  source 1..24: mol_type = other DNA
accggcgtcgtcggtcgcgattaa

SEQ ID NO: 18 - DNA, 24 bp, synthetic construct
  misc_feature 1..24: note = source = /note="Description of Artificial Sequence: Synthetic primer"
  source 1..24: mol_type = other DNA
aaacttaatcgcgaccgacgacgc

SEQ ID NO: 19 - DNA, 24 bp, synthetic construct
  misc_feature 1..24: note = source = /note="Description of Artificial Sequence: Synthetic primer"
  source 1..24: mol_type = other DNA
accggggtgatgttgcctgaccgg

SEQ ID NO: 20 - DNA, 24 bp, synthetic construct
  misc_feature 1..24: note = source = /note="Description of Artificial Sequence: Synthetic primer"
  source 1..24: mol_type = other DNA
aaacccggtcaggcaacatcaccc

SEQ ID NO: 21 - DNA, 21 bp, synthetic construct
  misc_feature 1..21: note = source = /note="Description of Artificial Sequence: Synthetic primer"
  source 1..21: mol_type = other DNA
ctttggccacgttgtgagaga

SEQ ID NO: 22 - DNA, 19 bp, synthetic construct
  misc_feature 1..19: note = source = /note="Description of Artificial Sequence: Synthetic primer"
  source 1..19: mol_type = other DNA
ggatgtttgcagcctgacg

SEQ ID NO: 23 - DNA, 23 bp, synthetic construct
  misc_feature 1..23: note = source = /note="Description of Artificial Sequence: Synthetic primer"
  source 1..23: mol_type = other DNA
gagtgcttttctcctacagtcac

SEQ ID NO: 24 - DNA, 20 bp, synthetic construct
  misc_feature 1..20: note = source = /note="Description of Artificial Sequence: Synthetic primer"
  source 1..20: mol_type = other DNA
ttcaagtagtcggggatgtc

SEQ ID NO: 25 - DNA, 53 bp, synthetic construct
  misc_feature 1..53: note = source = /note="Description of Artificial Sequence: Synthetic primer"
  source 1..53: mol_type = other DNA
tcgtcggcagcgtcagatgtgtataagagacagaaagcactaactccatctcc

SEQ ID NO: 26 - DNA, 54 bp, synthetic construct
  misc_feature 1..54: note = source = /note="Description of Artificial Sequence: Synthetic primer"
  source 1..54: mol_type = other DNA
gtctcgtgggctcggagatgtgtataagagacagacagccaccacggccaggat

SEQ ID NO: 27 - DNA, 52 bp, synthetic construct
  misc_feature 1..52: note = source = /note="Description of Artificial Sequence: Synthetic primer"
  source 1..52: mol_type = other DNA
tcgtcggcagcgtcagatgtgtataagagacagcattcatgcgtcttcacct

SEQ ID NO: 28 - DNA, 54 bp, synthetic construct
  misc_feature 1..54: note = source = /note="Description of Artificial Sequence: Synthetic primer"
  source 1..54: mol_type = other DNA
gtctcgtgggctcggagatgtgtataagagacagatattgtctttgtgttcccg

SEQ ID NO: 29 - DNA, 54 bp, synthetic construct
  misc_feature 1..54: note = source = /note="Description of Artificial Sequence: Synthetic primer"
  source 1..54: mol_type = other DNA
tcgtcggcagcgtcagatgtgtataagagacagttccagaaccggaggacaaag

SEQ ID NO: 30 - DNA, 54 bp, synthetic construct
  misc_feature 1..54: note = source = /note="Description of Artificial Sequence: Synthetic primer"
  source 1..54: mol_type = other DNA
gtctcgtgggctcggagatgtgtataagagacagccaccctagtcattggaggt

SEQ ID NO: 31 - DNA, 53 bp, synthetic construct
  misc_feature 1..53: note = source = /note="Description of Artificial Sequence: Synthetic primer"
  source 1..53: mol_type = other DNA
tcgtcggcagcgtcagatgtgtataagagacagaggcagagggtccaaagcag

SEQ ID NO: 32 - DNA, 54 bp, synthetic construct
  misc_feature 1..54: note = source = /note="Description of Artificial Sequence: Synthetic primer"
  source 1..54: mol_type = other DNA
gtctcgtgggctcggagatgtgtataagagacagatcagaagccctaagcggga

SEQ ID NO: 33 - DNA, 53 bp, synthetic construct
  misc_feature 1..53: note = source = /note="Description of Artificial Sequence: Synthetic primer"
  source 1..53: mol_type = other DNA
tcgtcggcagcgtcagatgtgtataagagacagctcccttttctccaggccac

SEQ ID NO: 34 - DNA, 54 bp, synthetic construct
  misc_feature 1..54: note = source = /note="Description of Artificial Sequence: Synthetic primer"
  source 1..54: mol_type = other DNA
gtctcgtgggctcggagatgtgtataagagacagatagtagttgctctggcggt

SEQ ID NO: 35 - DNA, 24 bp, synthetic construct
  misc_feature 1..24: note = source = /note="Description of Artificial Sequence: Synthetic primer"
  source 1..24: mol_type = other DNA
accgccttgtatttccgaagacat

SEQ ID NO: 36 - DNA, 24 bp, synthetic construct
  misc_feature 1..24: note = source = /note="Description of Artificial Sequence: Synthetic primer"
  source 1..24: mol_type = other DNA
accgtacaaggacttctgcatcca

SEQ ID NO: 37 - DNA, 24 bp, synthetic construct
  misc_feature 1..24: note = source = /note="Description of Artificial Sequence: Synthetic primer"
  source 1..24: mol_type = other DNA
accgtcacatatttgcattctcca

SEQ ID NO: 38 - DNA, 24 bp, synthetic construct
  misc_feature 1..24: note = source = /note="Description of Artificial Sequence: Synthetic primer"
  source 1..24: mol_type = other DNA
accgtggagaatgcaaatatgtga

SEQ ID NO: 39 - DNA, 24 bp, synthetic construct
  misc_feature 1..24: note = source = /note="Description of Artificial Sequence: Synthetic primer"
  source 1..24: mol_type = other DNA
accggcaaatatgtgaaggagctc

SEQ ID NO: 40 - DNA, 24 bp, synthetic construct
  misc_feature 1..24: note = source = /note="Description of Artificial Sequence: Synthetic primer"
  source 1..24: mol_type = other DNA
accgcaaatatgtgaaggagctcc

SEQ ID NO: 41 - DNA, 24 bp, synthetic construct
  misc_feature 1..24: note = source = /note="Description of Artificial Sequence: Synthetic primer"
  source 1..24: mol_type = other DNA
accgcttacatgcaggagggagcc

SEQ ID NO: 42 - DNA, 24 bp, synthetic construct
  misc_feature 1..24: note = source = /note="Description of Artificial Sequence: Synthetic primer"
  source 1..24: mol_type = other DNA
accgagctgccacccgggttacca

SEQ ID NO: 43 - DNA, 24 bp, synthetic construct
  misc_feature 1..24: note = source = /note="Description of Artificial Sequence: Synthetic primer"
  source 1..24: mol_type = other DNA
accgacccgggttaccatggagag

SEQ ID NO: 44 - DNA, 24 bp, synthetic construct
  misc_feature 1..24: note = source = /note="Description of Artificial Sequence: Synthetic primer"
  source 1..24: mol_type = other DNA
accgcacctctctccatggtaacc

SEQ ID NO: 45 - DNA, 24 bp, synthetic construct
  misc_feature 1..24: note = source = /note="Description of Artificial Sequence: Synthetic primer"
  source 1..24: mol_type = other DNA
accgaccatggagagaggtgtcat

SEQ ID NO: 46 - DNA, 24 bp, synthetic construct
  misc_feature 1..24: note = source = /note="Description of Artificial Sequence: Synthetic primer"
  source 1..24: mol_type = other DNA
accggcccatgacacctctctcca

SEQ ID NO: 47 - DNA, 24 bp, synthetic construct
  misc_feature 1..24: note = source = /note="Description of Artificial Sequence: Synthetic primer"
  source 1..24: mol_type = other DNA
accgtcatgggctgagcctcccag

SEQ ID NO: 48 - DNA, 24 bp, synthetic construct
  misc_feature 1..24: note = source = /note="Description of Artificial Sequence: Synthetic primer"
  source 1..24: mol_type = other DNA
accggtatataagcgattttccac

SEQ ID NO: 49 - DNA, 24 bp, synthetic construct
  misc_feature 1..24: note = source = /note="Description of Artificial Sequence: Synthetic primer"
  source 1..24: mol_type = other DNA
aaacatgtcttcggaaatacaagg

SEQ ID NO: 50 - DNA, 24 bp, synthetic construct
  misc_feature 1..24: note = source = /note="Description of Artificial Sequence: Synthetic primer"
  source 1..24: mol_type = other DNA
aaactggatgcagaagtccttgta

SEQ ID NO: 51 - DNA, 24 bp, synthetic construct
  misc_feature 1..24: note = source = /note="Description of Artificial Sequence: Synthetic primer"
  source 1..24: mol_type = other DNA
aaactggagaatgcaaatatgtga

SEQ ID NO: 52 - DNA, 24 bp, synthetic construct
  misc_feature 1..24: note = source = /note="Description of Artificial Sequence: Synthetic primer"
  source 1..24: mol_type = other DNA
aaactcacatatttgcattctcca

SEQ ID NO: 53 - DNA, 24 bp, synthetic construct
  misc_feature 1..24: note = source = /note="Description of Artificial Sequence: Synthetic primer"
  source 1..24: mol_type = other DNA
aaacgagctccttcacatatttgc

SEQ ID NO: 54 - DNA, 24 bp, synthetic construct
  misc_feature 1..24: note = source = /note="Description of Artificial Sequence: Synthetic primer"
  source 1..24: mol_type = other DNA
aaacggagctccttcacatatttg

SEQ ID NO: 55 - DNA, 24 bp, synthetic construct
  misc_feature 1..24: note = source = /note="Description of Artificial Sequence: Synthetic primer"
  source 1..24: mol_type = other DNA
aaacggctccctcctgcatgtaag

SEQ ID NO: 56 - DNA, 24 bp, synthetic construct
  misc_feature 1..24: note = source = /note="Description of Artificial Sequence: Synthetic primer"
  source 1..24: mol_type = other DNA
aaactggtaacccgggtggcagct

SEQ ID NO: 57 - DNA, 24 bp, synthetic construct
  misc_feature 1..24: note = source = /note="Description of Artificial Sequence: Synthetic primer"
  source 1..24: mol_type = other DNA
aaacctctccatggtaacccgggt

SEQ ID NO: 58 - DNA, 24 bp, synthetic construct
  misc_feature 1..24: note = source = /note="Description of Artificial Sequence: Synthetic primer"
  source 1..24: mol_type = other DNA
aaacggttaccatggagagaggtg

SEQ ID NO: 59 - DNA, 24 bp, synthetic construct
  misc_feature 1..24: note = source = /note="Description of Artificial Sequence: Synthetic primer"
  source 1..24: mol_type = other DNA
aaacatgacacctctctccatggt

SEQ ID NO: 60 - DNA, 24 bp, synthetic construct
  misc_feature 1..24: note = source = /note="Description of Artificial Sequence: Synthetic primer"
  source 1..24: mol_type = other DNA
aaactggagagaggtgtcatgggc

SEQ ID NO: 61 - DNA, 24 bp, synthetic construct
  misc_feature 1..24: note = source = /note="Description of Artificial Sequence: Synthetic primer"
  source 1..24: mol_type = other DNA
aaacctgggaggctcagcccatga

SEQ ID NO: 62 - DNA, 24 bp, synthetic construct
  misc_feature 1..24: note = source = /note="Description of Artificial Sequence: Synthetic primer"
  source 1..24: mol_type = other DNA
aaacgtggaaaatcgcttatatac

SEQ ID NO: 63 - DNA, 24 bp, synthetic construct
  misc_feature 1..24: note = source = /note="Description of Artificial Sequence: Synthetic primer"
  source 1..24: mol_type = other DNA
accgcaggttccacgggatgctct

SEQ ID NO: 64 - DNA, 24 bp, synthetic construct
  misc_feature 1..24: note = source = /note="Description of Artificial Sequence: Synthetic primer"
  source 1..24: mol_type = other DNA
aaacagagcatcccgtggaacctg

SEQ ID NO: 65 - DNA, 24 bp, synthetic construct
  misc_feature 1..24: note = source = /note="Description of Artificial Sequence: Synthetic primer"
  source 1..24: mol_type = other DNA
accggagtccgagcagaagaagaa

SEQ ID NO: 66 - DNA, 24 bp, synthetic construct
  misc_feature 1..24: note = source = /note="Description of Artificial Sequence: Synthetic primer"
  source 1..24: mol_type = other DNA
aaacttcttcttctgctcggactc

SEQ ID NO: 67 - DNA, 24 bp, synthetic construct
  misc_feature 1..24: note = source = /note="Description of Artificial Sequence: Synthetic primer"
  source 1..24: mol_type = other DNA
accgaatcacccaggcggtgtagt

SEQ ID NO: 68 - DNA, 24 bp, synthetic construct
  misc_feature 1..24: note = source = /note="Description of Artificial Sequence: Synthetic primer"
  source 1..24: mol_type = other DNA
aaacactacaccgcctgggtgatt

SEQ ID NO: 69 - DNA, 23 bp, synthetic construct
  misc_feature 1..23: note = source = /note="Description of Artificial Sequence: Synthetic primer"
  source 1..23: mol_type = other DNA
accggcactgcggctggaggtgg

SEQ ID NO: 70 - DNA, 23 bp, synthetic construct
  misc_feature 1..23: note = source = /note="Description of Artificial Sequence: Synthetic primer"
  source 1..23: mol_type = other DNA
aaacccacctccagccgcagtgc

SEQ ID NO: 71 - DNA, 24 bp, synthetic construct
  misc_feature 1..24: note = source = /note="Description of Artificial Sequence: Synthetic primer"
  source 1..24: mol_type = other DNA
accggcgtcgtcggtcgcgattaa

SEQ ID NO: 72 - DNA, 24 bp, synthetic construct
  misc_feature 1..24: note = source = /note="Description of Artificial Sequence: Synthetic primer"
  source 1..24: mol_type = other DNA
aaacttaatcgcgaccgacgacgc

SEQ ID NO: 73 - DNA, 24 bp, synthetic construct
  misc_feature 1..24: note = source = /note="Description of Artificial Sequence: Synthetic primer"
  source 1..24: mol_type = other DNA
accgggggttccagggcctgtctg

SEQ ID NO: 74 - DNA, 24 bp, synthetic construct
  misc_feature 1..24: note = source = /note="Description of Artificial Sequence: Synthetic primer"
  source 1..24: mol_type = other DNA
aaaccagacaggccctggaacccc

SEQ ID NO: 75 - DNA, 24 bp, synthetic construct
  misc_feature 1..24: note = source = /note="Description of Artificial Sequence: Synthetic primer"
  source 1..24: mol_type = other DNA
accgggcccagcctgctgtggtac

SEQ ID NO: 76 - DNA, 24 bp, synthetic construct
  misc_feature 1..24: note = source = /note="Description of Artificial Sequence: Synthetic primer"
  source 1..24: mol_type = other DNA
aaacgtaccacagcaggctgggcc

SEQ ID NO: 77 - DNA, 24 bp, synthetic construct
  misc_feature 1..24: note = source = /note="Description of Artificial Sequence: Synthetic primer"
  source 1..24: mol_type = other DNA
accgcaatgtcaatgcacaagctc

SEQ ID NO: 78 - DNA, 24 bp, synthetic construct
  misc_feature 1..24: note = source = /note="Description of Artificial Sequence: Synthetic primer"
  source 1..24: mol_type = other DNA
aaacgagcttgtgcattgacattg

SEQ ID NO: 79 - DNA, 24 bp, synthetic construct
  misc_feature 1..24: note = source = /note="Description of Artificial Sequence: Synthetic primer"
  source 1..24: mol_type = other DNA
accggtggaccaagcgagccttcc

SEQ ID NO: 80 - DNA, 24 bp, synthetic construct
  misc_feature 1..24: note = source = /note="Description of Artificial Sequence: Synthetic primer"
  source 1..24: mol_type = other DNA
aaacggaaggctcgcttggtccac

SEQ ID NO: 81 - DNA, 24 bp, synthetic construct
  misc_feature 1..24: note = source = /note="Description of Artificial Sequence: Synthetic primer"
  source 1..24: mol_type = other DNA
accggcttacttggaatgtttact

SEQ ID NO: 82 - DNA, 24 bp, synthetic construct
  misc_feature 1..24: note = source = /note="Description of Artificial Sequence: Synthetic primer"
  source 1..24: mol_type = other DNA
aaacagtaaacattccaagtaagc

SEQ ID NO: 83 - DNA, 24 bp, synthetic construct
  misc_feature 1..24: note = source = /note="Description of Artificial Sequence: Synthetic primer"
  source 1..24: mol_type = other DNA
accgttcatgagtcttgacaacaa

SEQ ID NO: 84 - DNA, 24 bp, synthetic construct
  misc_feature 1..24: note = source = /note="Description of Artificial Sequence: Synthetic primer"
  source 1..24: mol_type = other DNA
aaacttgttgtcaagactcatgaa

SEQ ID NO: 85 - DNA, 24 bp, synthetic construct
  misc_feature 1..24: note = source = /note="Description of Artificial Sequence: Synthetic primer"
  source 1..24: mol_type = other DNA
accggggtgatgttgcctgaccgg

SEQ ID NO: 86 - DNA, 24 bp, synthetic construct
  misc_feature 1..24: note = source = /note="Description of Artificial Sequence: Synthetic primer"
  source 1..24: mol_type = other DNA
aaacccggtcaggcaacatcaccc

SEQ ID NO: 87 - DNA, 20 bp, synthetic construct
  misc_feature 1..20: note = source = /note="Description of Artificial Sequence: Synthetic primer"
  source 1..20: mol_type = other DNA
gaccgagatagggttgagtg

SEQ ID NO: 88 - DNA, 20 bp, synthetic construct
  misc_feature 1..20: note = source = /note="Description of Artificial Sequence: Synthetic primer"
  source 1..20: mol_type = other DNA
caccccaggctttacccgaa

SEQ ID NO: 89 - DNA, 18 bp, synthetic construct
  misc_feature 1..18: note = source = /note="Description of Artificial Sequence: Synthetic primer"
  source 1..18: mol_type = other DNA
gcgtccatgtcttcggaa

SEQ ID NO: 90 - DNA, 20 bp, synthetic construct
  misc_feature 1..20: note = source = /note="Description of Artificial Sequence: Synthetic primer"
  source 1..20: mol_type = other DNA
ataaggcctctcaaccacac

SEQ ID NO: 91 - DNA, 59 bp, synthetic construct
  misc_feature 1..59: note = source = /note="Description of Artificial Sequence: Synthetic primer"
  source 1..59: mol_type = other DNA
cgttgtaaaacgacggccagtcccccggtcaggcaacagaacccgagcgcgacgtaata

SEQ ID NO: 92 - DNA, 58 bp, synthetic construct
  misc_feature 1..58: note = source = /note="Description of Artificial Sequence: Synthetic primer"
  source 1..58: mol_type = other DNA
catgttaatgcagctggcacatgttgcctgaccgggggataaggcctctcaaccacac

SEQ ID NO: 93 - DNA, 18 bp, synthetic construct
  misc_feature 1..18: note = source = /note="Description of Artificial Sequence: Synthetic primer"
  source 1..18: mol_type = other DNA
gcgtccatgtcttcggaa

SEQ ID NO: 94 - DNA, 20 bp, synthetic construct
  misc_feature 1..20: note = source = /note="Description of Artificial Sequence: Synthetic primer"
  source 1..20: mol_type = other DNA
ataaggcctctcaaccacac

SEQ ID NO: 95 - DNA, 53 bp, synthetic construct
  misc_feature 1..53: note = source = /note="Description of Artificial Sequence: Synthetic primer"
  source 1..53: mol_type = other DNA
tcgtcggcagcgtcagatgtgtataagagacagcgggaaaagaaagaagaaag

SEQ ID NO: 96 - DNA, 54 bp, synthetic construct
  misc_feature 1..54: note = source = /note="Description of Artificial Sequence: Synthetic primer"
  source 1..54: mol_type = other DNA
gtctcgtgggctcggagatgtgtataagagacagacaaagtgtgctgatgagat

SEQ ID NO: 97 - DNA, 53 bp, synthetic construct; identical to SEQ ID NO: 25
  misc_feature 1..53: note = source = /note="Description of Artificial Sequence: Synthetic primer"
  source 1..53: mol_type = other DNA

SEQ ID NO: 98 - DNA, 54 bp, synthetic construct; identical to SEQ ID NO: 26
  misc_feature 1..54: note = source = /note="Description of Artificial Sequence: Synthetic primer"
  source 1..54: mol_type = other DNA

SEQ ID NO: 99 - DNA, 53 bp, synthetic construct
  misc_feature 1..53: note = source = /note="Description of Artificial Sequence: Synthetic primer"
  source 1..53: mol_type = other DNA
tcgtcggcagcgtcagatgtgtataagagacagatgtggggacaggtttgatc

SEQ ID NO: 100 - DNA, 54 bp, synthetic construct
  misc_feature 1..54: note = source = /note="Description of Artificial Sequence: Synthetic primer"
  source 1..54: mol_type = other DNA
gtctcgtgggctcggagatgtgtataagagacagtggtattcatccgcccggta

SEQ ID NO: 101 - DNA, 52 bp, synthetic construct; identical to SEQ ID NO: 27
  misc_feature 1..52: note = source = /note="Description of Artificial Sequence: Synthetic primer"
  source 1..52: mol_type = other DNA

SEQ ID NO: 102 - DNA, 54 bp, synthetic construct; identical to SEQ ID NO: 28
  misc_feature 1..54: note = source = /note="Description of Artificial Sequence: Synthetic primer"
  source 1..54: mol_type = other DNA

SEQ ID NO: 103 - DNA, 54 bp, synthetic construct; identical to SEQ ID NO: 29
  misc_feature 1..54: note = source = /note="Description of Artificial Sequence: Synthetic primer"
  source 1..54: mol_type = other DNA

SEQ ID NO: 104 - DNA, 54 bp, synthetic construct; identical to SEQ ID NO: 30
  misc_feature 1..54: note = source = /note="Description of Artificial Sequence: Synthetic primer"
  source 1..54: mol_type = other DNA

SEQ ID NO: 105 - DNA, 53 bp, synthetic construct; identical to SEQ ID NO: 31
  misc_feature 1..53: note = source = /note="Description of Artificial Sequence: Synthetic primer"
  source 1..53: mol_type = other DNA

SEQ ID NO: 106 - DNA, 54 bp, synthetic construct; identical to SEQ ID NO: 32
  misc_feature 1..54: note = source = /note="Description of Artificial Sequence: Synthetic primer"
  source 1..54: mol_type = other DNA

SEQ ID NO: 107 - DNA, 53 bp, synthetic construct; identical to SEQ ID NO: 33
  misc_feature 1..53: note = source = /note="Description of Artificial Sequence: Synthetic primer"
  source 1..53: mol_type = other DNA

SEQ ID NO: 108 - DNA, 54 bp, synthetic construct; identical to SEQ ID NO: 34
  misc_feature 1..54: note = source = /note="Description of Artificial Sequence: Synthetic primer"
  source 1..54: mol_type = other DNA

SEQ ID NO: 109 - DNA, 53 bp, synthetic construct
  misc_feature 1..53: note = source = /note="Description of Artificial Sequence: Synthetic primer"
  source 1..53: mol_type = other DNA
tcgtcggcagcgtcagatgtgtataagagacaggccccctgtcatggcatctt

SEQ ID NO: 110 - DNA, 57 bp, synthetic construct
  misc_feature 1..57: note = source = /note="Description of Artificial Sequence: Synthetic primer"
  source 1..57: mol_type = other DNA
gtctcgtgggctcggagatgtgtataagagacaggtgggggttagacccaatatcag

SEQ ID NO: 111 - DNA, 53 bp, synthetic construct
  misc_feature 1..53: note = source = /note="Description of Artificial Sequence: Synthetic primer"
  source 1..53: mol_type = other DNA
tcgtcggcagcgtcagatgtgtataagagacagcccttcctcacctctctcca

SEQ ID NO: 112 - DNA, 54 bp, synthetic construct
  misc_feature 1..54: note = source = /note="Description of Artificial Sequence: Synthetic primer"
  source 1..54: mol_type = other DNA
gtctcgtgggctcggagatgtgtataagagacagcacgaagctctccgatgtgt

SEQ ID NO: 113 - DNA, 53 bp, synthetic construct
  misc_feature 1..53: note = source = /note="Description of Artificial Sequence: Synthetic primer"
  source 1..53: mol_type = other DNA
tcgtcggcagcgtcagatgtgtataagagacagtagaaggcagaagggcttgc

SEQ ID NO: 114 - DNA, 54 bp, synthetic construct
  misc_feature 1..54: note = source = /note="Description of Artificial Sequence: Synthetic primer"
  source 1..54: mol_type = other DNA
gtctcgtgggctcggagatgtgtataagagacagagtggctttgcctggagatg

SEQ ID NO: 115 - DNA, 55 bp, synthetic construct
  misc_feature 1..55: note = source = /note="Description of Artificial Sequence: Synthetic primer"
  source 1..55: mol_type = other DNA
tcgtcggcagcgtcagatgtgtataagagacagagcgggtcactctatatgctct

SEQ ID NO: 116 - DNA, 55 bp, synthetic construct
  misc_feature 1..55: note = source = /note="Description of Artificial Sequence: Synthetic primer"
  source 1..55: mol_type = other DNA
gtctcgtgggctcggagatgtgtataagagacagtggtagtcacagaagggacac

SEQ ID NO: 117 - DNA, 55 bp, synthetic construct
  misc_feature 1..55: note = source = /note="Description of Artificial Sequence: Synthetic primer"
  source 1..55: mol_type = other DNA
tcgtcggcagcgtcagatgtgtataagagacagaaacaagtgacacctcaacctg

SEQ ID NO: 118 - DNA, 55 bp, synthetic construct
  misc_feature 1..55: note = source = /note="Description of Artificial Sequence: Synthetic primer"
  source 1..55: mol_type = other DNA
gtctcgtgggctcggagatgtgtataagagacagcgctagcaggagttagctgga

SEQ ID NO: 119 - DNA, 56 bp, synthetic construct
  misc_feature 1..56: note = source = /note="Description of Artificial Sequence: Synthetic primer"
  source 1..56: mol_type = other DNA
gtctcgtgggctcggagatgtgtataagagacagagtgcagactctggagccctga

SEQ ID NO: 120 - DNA, 55 bp, synthetic construct
  misc_feature 1..55: note = source = /note="Description of Artificial Sequence: Synthetic primer"
  source 1..55: mol_type = other DNA
tcgtcggcagcgtcagatgtgtataagagacagctgtaggccctgaagttgcccc

SEQ ID NO: 121 - DNA, 23 bp, synthetic construct
  misc_feature 1..23: note = source = /note="Description of Artificial Sequence: Synthetic primer"
  source 1..23: mol_type = other DNA
gagtgcttttctcctacagtcac

SEQ ID NO: 122 - DNA, 20 bp, synthetic construct
  misc_feature 1..20: note = source = /note="Description of Artificial Sequence: Synthetic primer"
  source 1..20: mol_type = other DNA
ttcaagtagtcggggatgtc

SEQ ID NO: 123 - DNA, 21 bp, synthetic construct
  misc_feature 1..21: note = source = /note="Description of Artificial Sequence: Synthetic primer"
  source 1..21: mol_type = other DNA
ctttggccacgttgtgagaga

SEQ ID NO: 124 - DNA, 19 bp, synthetic construct
  misc_feature 1..19: note = source = /note="Description of Artificial Sequence: Synthetic primer"
  source 1..19: mol_type = other DNA
ggatgtttgcagcctgacg

SEQ ID NO: 125 - DNA, 154 bp, synthetic construct
  misc_feature 1..154: note = source = /note="Description of Artificial Sequence: Synthetic polynucleotide"
  source 1..154: mol_type = other DNA
tttgtagaaacatttgaaaatgttccctgggtaggtaactctggggtagcagtaccgttggtttaattgagttgcaattggttaataacggtatttgtcaagactcatgaacccagaagctatagggaaacgaggaggaagaatcagaacctaa

SEQ ID NO: 126 - DNA, 95 bp, synthetic construct
  misc_feature 1..95: note = source = /note="Description of Artificial Sequence: Synthetic oligonucleotide"
  source 1..95: mol_type = other DNA
ttattaggatatttttattttttattttttttttttttttttggataattattattttattatttattttttttttattaaatattttaaggata

SEQ ID NO: 127 - protein, 36 aa, unidentified
  MOD_RES 2: note = Any amino acid
  MOD_RES 4..29: note = Any amino acid
  SITE 4..29: note = /note="This region may encompass 23-26 Xaa residues, wherein Xaa is any amino acid"
  MOD_RES 32..35: note = Any amino acid
  SITE 32..35: note = /note="This region may encompass 2-4 Xaa residues, wherein Xaa is any amino acid"
  REGION 1..36: note = source = /note="Description of Unknown: Zinc-coordinating motif"
HXEXXXXXXXXXXXXXXXXXXXXXXXXXXPCXXXXC

SEQ ID NO: 128-129 - skipped (2 entries)

SEQ ID NO: 130 - protein, 208 aa, Mus sp.
MKLLPSVMLKLFLAAVLSALVTGESLERLRRGLAAATSNPDPPTGSTNQLLPTGGDRAQGVQDLEGTDLNLFKVAFSSKPQGLATPSKERNGKKKKKGKGLGKKRDPCLRKYKDYCIHGECRYLQEFRTPSCKCLPGYHGHRCHGLTLPVENPLYTYDHTTVLAVVAVVLSSVCLLVIVGLLMFRYHRRGGYDLESEEKVKLGVASSH

SEQ ID NO: 131 - DNA, 20 bp, synthetic construct
  misc_feature 1..20: note = source = /note="Description of Artificial Sequence: Synthetic oligonucleotide"
  source 1..20: mol_type = other DNA
ggttaccatggagagaggtg

SEQ ID NO: 132 - DNA, 20 bp, synthetic construct
  misc_feature 1..20: note = source = /note="Description of Artificial Sequence: Synthetic oligonucleotide"
  source 1..20: mol_type = other DNA
cacctctctccatggtaacc

SEQ ID NO: 133 - protein, 10 aa, synthetic construct
  REGION 1..10: note = source = /note="Description of Artificial Sequence: Synthetic peptide"
CHPGYHGKRC

SEQ ID NO: 134 - protein, 10 aa, synthetic construct
  REGION 1..10: note = source = /note="Description of Artificial Sequence: Synthetic peptide"
CHPGYHGKKC

SEQ ID NO: 135 - protein, 10 aa, synthetic construct
  REGION 1..10: note = source = /note="Description of Artificial Sequence: Synthetic peptide"
CHPGYHEKKC

SEQ ID NO: 136 - protein, 10 aa, synthetic construct
  REGION 1..10: note = source = /note="Description of Artificial Sequence: Synthetic peptide"
CHPGYHKKKC

SEQ ID NO: 137 - DNA, 20 bp, synthetic construct
  misc_feature 1..20: note = source = /note="Description of Artificial Sequence: Synthetic oligonucleotide"
  source 1..20: mol_type = other DNA
agagcatcccgtggaacctg

SEQ ID NO: 138 - DNA, 20 bp, synthetic construct
  misc_feature 1..20: note = source = /note="Description of Artificial Sequence: Synthetic oligonucleotide"
  source 1..20: mol_type = other DNA
caggttccacgggatgctct

SEQ ID NO: 139 - DNA, 20 bp, synthetic construct
  misc_feature 1..20: note = source = /note="Description of Artificial Sequence: Synthetic oligonucleotide"
  source 1..20: mol_type = other DNA
aatcacccaggcggtgtagt

SEQ ID NO: 140 - DNA, 20 bp, synthetic construct
  misc_feature 1..20: note = source = /note="Description of Artificial Sequence: Synthetic oligonucleotide"
  source 1..20: mol_type = other DNA
atcacgcagctcatgccctt

SEQ ID NO: 141 - DNA, 20 bp, synthetic construct
  misc_feature 1..20: note = source = /note="Description of Artificial Sequence: Synthetic oligonucleotide"
  source 1..20: mol_type = other DNA
gagtccgagcagaagaagaa

SEQ ID NO: 142 - DNA, 20 bp, synthetic construct
  misc_feature 1..20: note = source = /note="Description of Artificial Sequence: Synthetic oligonucleotide"
  source 1..20: mol_type = other DNA
ggcactgcggctggaggtgg

SEQ ID NO: 143 - DNA, 153 bp, Homo sapiens
  source 1..153: mol_type = genomic DNA
ccatgtcttcggaaatacaaggacttctgcatccatggagaatgcaaatatgtgaaggagctccgggctccctcctgcatctgccacccgggttaccatggagagaggtgtcatgggctgagcctcccagtggaaaatcgcttatatacctat

SEQ ID NO: 144 - protein, 51 aa, Homo sapiens
PCLRKYKDFCIHGECKYVKELRAPSCICHPGYHGERCHGLSLPVENRLYTY

SEQ ID NO: 145 - protein, 51 aa, Mus sp.
PCLRKYKDYCIHGECRYLQEFRTPSCKCLPGYHGHRCHGLTLPVENPLYTY

SEQ ID NO: 146 - DNA, 39 bp, Homo sapiens
  source 1..39: mol_type = other DNA
tgccacccgggttaccatggagagaggtgtcatgggctg

SEQ ID NO: 147 - protein, 13 aa, Homo sapiens
CHPGYHGERCHGL

SEQ ID NO: 148 - DNA, 39 bp, synthetic construct
  misc_feature 1..39: note = source = /note="Description of Artificial Sequence: Synthetic oligonucleotide"
  source 1..39: mol_type = other DNA
tgccacccgggttaccatggaaaaaggtgtcatgggctg

SEQ ID NO: 149 - protein, 13 aa, synthetic construct
  REGION 1..13: note = source = /note="Description of Artificial Sequence: Synthetic peptide"
CHPGYHGKRCHGL

SEQ ID NO: 150 - DNA, 39 bp, synthetic construct
  misc_feature 1..39: note = source = /note="Description of Artificial Sequence: Synthetic oligonucleotide"
  source 1..39: mol_type = other DNA
tgccacccgggttaccatggaaaaaaatgtcatgggctg

SEQ ID NO: 151 - protein, 13 aa, synthetic construct
  REGION 1..13: note = source = /note="Description of Artificial Sequence: Synthetic peptide"
CHPGYHGKKCHGL

SEQ ID NO: 152 - DNA, 39 bp, synthetic construct
  misc_feature 1..39: note = source = /note="Description of Artificial Sequence: Synthetic oligonucleotide"
  source 1..39: mol_type = other DNA
tgccacccgggttaccatgaaaaaaaatgtcatgggctg

SEQ ID NO: 153 - protein, 13 aa, synthetic construct
  REGION 1..13: note = source = /note="Description of Artificial Sequence: Synthetic peptide"
CHPGYHEKKCHGL

SEQ ID NO: 154 - DNA, 39 bp, synthetic construct
  misc_feature 1..39: note = source = /note="Description of Artificial Sequence: Synthetic oligonucleotide"
  source 1..39: mol_type = other DNA
tgccacccgggttaccatggaaaaaagtgtcatgggctg

SEQ ID NO: 155 - DNA, 39 bp, synthetic construct
  misc_feature 1..39: note = source = /note="Description of Artificial Sequence: Synthetic oligonucleotide"
  source 1..39: mol_type = other DNA
tgccacccgggttaccataaaaaaaaatgtcatgggctg

SEQ ID NO: 156 - protein, 13 aa, synthetic construct
  REGION 1..13: note = source = /note="Description of Artificial Sequence: Synthetic peptide"
CHPGYHKKKCHGL

SEQ ID NO: 157 - DNA, 39 bp, Homo sapiens
  source 1..39: mol_type = other DNA
catggagaatgcaaatatgtgaaggagctccgggctccc

SEQ ID NO: 158 - protein, 13 aa, Homo sapiens
HGECKYVKELRAP

SEQ ID NO: 159 - DNA, 39 bp, synthetic construct
  misc_feature 1..39: note = source = /note="Description of Artificial Sequence: Synthetic oligonucleotide"
  source 1..39: mol_type = other DNA
catggagaatgcaaatgtgtgaaggagctccgggctccc

SEQ ID NO: 160 - protein, 13 aa, synthetic construct
  REGION 1..13: note = source = /note="Description of Artificial Sequence: Synthetic peptide"
HGECKCVKELRAP

SEQ ID NO: 161 - DNA, 39 bp, synthetic construct
  misc_feature 1..39: note = source = /note="Description of Artificial Sequence: Synthetic oligonucleotide"
  source 1..39: mol_type = other DNA
catggagaatgcaagtgtgtgaaggagctccgggctccc

SEQ ID NO: 162 - DNA, 39 bp, synthetic construct
  misc_feature 1..39: note = source = /note="Description of Artificial Sequence: Synthetic oligonucleotide"
  source 1..39: mol_type = other DNA
catggagaatgcaggtgtgtgaaggagctccgggctccc

SEQ ID NO: 163 - protein, 13 aa, synthetic construct
  REGION 1..13: note = source = /note="Description of Artificial Sequence: Synthetic peptide"
HGECRCVKELRAP

SEQ ID NO: 164 - DNA, 39 bp, synthetic construct
  misc_feature 1..39: note = source = /note="Description of Artificial Sequence: Synthetic oligonucleotide"
  source 1..39: mol_type = other DNA
catggagaatgcgaatgtgtgaaggagctccgggctccc

SEQ ID NO: 165 - protein, 13 aa, synthetic construct
  REGION 1..13: note = source = /note="Description of Artificial Sequence: Synthetic peptide"
HGECECVKELRAP

SEQ ID NO: 166 - DNA, 39 bp, synthetic construct
  misc_feature 1..39: note = source = /note="Description of Artificial Sequence: Synthetic oligonucleotide"
  source 1..39: mol_type = other DNA
catggagaatgcagatgtgtgaaggagctccgggctccc

SEQ ID NO: 167 - protein, 11 aa, Homo sapiens
CIHGECKYVKE

SEQ ID NO: 168 - protein, 8 aa, Homo sapiens
GYHGERCH

SEQ ID NO: 169 - protein, 11 aa, Pan sp.
CIHGECKYVKE

SEQ ID NO: 170 - protein, 8 aa, Pan sp.
GYHGERCH

SEQ ID NO: 171 - protein, 11 aa, unidentified
  REGION 1..11: note = source = /note="Description of Unknown: Monkey HBEGF sequence"
CIHGECKYVKE

SEQ ID NO: 172 - protein, 8 aa, unidentified
  REGION 1..8: note = source = /note="Description of Unknown: Monkey HBEGF sequence"
GYHGERCH

SEQ ID NO: 173 - protein, 11 aa, unidentified
  REGION 1..11: note = source = /note="Description of Unknown: Hamster HBEGF sequence"
CIHGECKYLKD

SEQ ID NO: 174 - protein, 8 aa, unidentified
  REGION 1..8: note = source = /note="Description of Unknown: Hamster HBEGF sequence"
GYHGERCH

SEQ ID NO: 175 - protein, 11 aa, Sus sp.
CIHGECKYVKE

SEQ ID NO: 176 - protein, 8 aa, Sus sp.
GYHGERCH

SEQ ID NO: 177 - protein, 11 aa, unidentified
  REGION 1..11: note = source = /note="Description of Unknown: Rabbit HBEGF sequence"
CIHGECKYLKE

SEQ ID NO: 178 - protein, 8 aa, unidentified
  REGION 1..8: note = source = /note="Description of Unknown: Rabbit HBEGF sequence"
GYHGERCH

SEQ ID NO: 179 - protein, 11 aa, Rattus sp.
CIHGECRYLKE

SEQ ID NO: 180 - protein, 8 aa, Rattus sp.
GYHGQRCH

SEQ ID NO: 181 - protein, 11 aa, Mus sp.
CIHGECRYLQE

SEQ ID NO: 182 - protein, 8 aa, Mus sp.
GYHGHRCH

SEQ ID NO: 183 - protein, 11 aa, Gallus gallus
CIHGECKYIRE

SEQ ID NO: 184 - protein, 8 aa, Gallus gallus
GYHGERCH

SEQ ID NO: 185 - protein, 11 aa, Danio rerio
CIHGVCHYLRD

SEQ ID NO: 186 - protein, 8 aa, Danio rerio
GYSGERCH

SEQ ID NO: 187 - protein, 208 aa, Homo sapiens; identical to SEQ ID NO: 8